European Patent Application EP 4 458 988 A2, published November 6, 2024. Title: ASSAY FOR PRE-OPERATIVE PREDICTION OF ORGAN FUNCTION RECOVERY. Applicant: The Regents of the University of California. Application US PCTUS1840961, filed July 5, 2018. The sequence listing filed with the application follows.

SEQUENCE LISTING (10 sequences)

SEQ ID NO: 1 - DNA, 19 bp, synthetic construct
  misc_feature 1..19: note = primer
  source 1..19: mol_type = other DNA
ccactcctccacctttgac

SEQ ID NO: 2 - DNA, 18 bp, synthetic construct
  misc_feature 1..18: note = primer
  source 1..18: mol_type = other DNA
accctgttgctgtagcca

SEQ ID NO: 3 - DNA, 20 bp, synthetic construct
  misc_feature 1..20: note = primer
  source 1..20: mol_type = other DNA
acccactgcctgtttctgtc

SEQ ID NO: 4 - DNA, 20 bp, synthetic construct
  misc_feature 1..20: note = primer
  source 1..20: mol_type = other DNA
atcacagcatgcaggtgtct

SEQ ID NO: 5 - DNA, 20 bp, synthetic construct
  misc_feature 1..20: note = primer
  source 1..20: mol_type = other DNA
caggacacctgggttcacac

SEQ ID NO: 6 - DNA, 20 bp, synthetic construct
  misc_feature 1..20: note = primer
  source 1..20: mol_type = other DNA
ggttggactcgatgaagagg

SEQ ID NO: 7 - DNA, 20 bp, synthetic construct
  misc_feature 1..20: note = primer
  source 1..20: mol_type = other DNA
aaaggcagctgaagaagcag

SEQ ID NO: 8 - DNA, 21 bp, synthetic construct
  misc_feature 1..21: note = primer
  source 1..21: mol_type = other DNA
tctttttccagagactcgtgc

SEQ ID NO: 9 - DNA, 20 bp, synthetic construct
  misc_feature 1..20: note = primer
  source 1..20: mol_type = other DNA
ctcagccaggaaggattttg

SEQ ID NO: 10 - DNA, 20 bp, synthetic construct
  misc_feature 1..20: note = primer
  source 1..20: mol_type = other DNA
tgataggctgcttggcagat